European Patent Specification EP 3 947 615 B1, published April 5, 2023. Title: Verwendung von Mannanase-Enzym in Kombination mit Catecholderivaten. Applicant: Henkel AG & Co. KGaA. The sequence listing filed with the application follows.

SEQUENCE LISTING (2 sequences)

SEQ ID NO: 1 - protein, 490 aa, Bacillus sp.
LNNGFKKIFSITLSLLLASSILFVSGTSTANANSGFYVSGTTLYDANGNPFVMRGINHGHAWYKDQATTAIEGIANTGANTVRIVLSDGGQWTKDDIHTVRNLISLAEDNHLVAVPEVHDATGYDSIASLNRAVDYWIEMRSALIGKEDTVIINIANEWFGSWEGDAWADGYKQAIPRLRNAGLNHTLMVDAAGWGQFPQSIHDYGREVFNADPQRNTMFSIHMYEYAGGNASQVRTNIDRVLNQDLALVIGEFGHRHTNGDVDEATIMSYSEQRGVGWLAWSWKGNGPEWEYLDLSNDWAGNNLTAWGNTIVNGPYGLRETSRLSTVFTGGGSDGGTSPTTLYDFEGSMQGWTGSSLSGGPWAVTEWSSKGSHSLKADIQLSSNSQHYLHVIQNTSLQQNSRIQATVKHANWGSVGNGMTARLYVKTGHGYTWYSGSFVPINGSSGTTLSLDLSNVQNLSQVREIGVQFQSASDSSGQTSIYIDNVIVE

SEQ ID NO: 2 - protein, 297 aa, Paenibacillus sp.
MATGFYVSGNKLYDSTGKPFVMRGVNHGHSWFKNDLNTAIPAIAKTGANTVRIVLSNGSLYTKDDLNAVKNIINVVNQNKMIAVLEVHDATGKDDYNSLDAAVNYWISIKEALIGKEDRVIVNIANEWYGTWNGSAWADGYKKAIPKLRNAGIKNTLIVDAAGWGQFPQSIVDYGQSVFAADSQKNTVFSIHMYEYAGKDAATVKANMENVLNKGLALIIGEFGGYHTNGDVDEYAIMRYGQEKGVGWLAWSWYGNSSGLNYLDMATGPNGSLTSFGNTVVNDTYGIKNTSQKAGIF